European Patent Application EP 4 190 358 A1, published June 7, 2023. Title: POLYPEPTIDE AS CARRIER FOR INTESTINAL BARRIER CROSSING. Applicant: AFFILOGIC. The sequence listing filed with the application follows.

SEQUENCE LISTING (80 sequences)

SEQ ID NO: 1 - protein, 66 aa, Sulfolobus acidocaldarius
MVKVKFKYKGEEKEVDTSKIKKVWRVGKMVSFTYDDNGKTGRGAVSEKDAPKELLDMLARAEREKK

SEQ ID NO: 2 - protein, 64 aa, Sulfolobus solfataricus
MATVKFKYKGEEKEVDISKIKKVWRVGKMISFTYDEGGGKTGRGAVSEKDAPKELLQMLEKQKK

SEQ ID NO: 3 - protein, 65 aa, Sulfolobus acidocaldarius
MAKVRFKYKGEEKEVDTSKIKKVWRVGKMVSFTYDDNGKTGRGAVSEKDAPKELMDMLARAEKKK

SEQ ID NO: 4 - protein, 64 aa, Sulfolobus shibatae
MVTVKFKYKGEEKEVDTSKIKKVWRVGKMISFTYDEGGGKTGRGAVSEKDAPKELLQMLEKQKK

SEQ ID NO: 5 - protein, 64 aa, Sulfolobus shibatae
MATVKFKYKGEEKQVDISKIKKVWRVGKMISFTYDEGGGKTGRGAVSEKDAPKELLQMLEKQKK

SEQ ID NO: 6 - protein, 64 aa, Sulfolobus tokodaii
MVTVKFKYKGEEKEVDISKIKKVWRVGKMISFTYDDNGKTGRGAVSEKDAPKELLQMLEKSGKK

SEQ ID NO: 7 - protein, 64 aa, Sulfolobus islandicus
MVTVKFKYKGEEKQVDTSKIKKVWRVGKMISFTYDEGGGKTGRGAVSEKDAPKELLQMLEKQKK

SEQ ID NO: 8 - protein, 64 aa, Sulfolobus islandicus
MTTVKFKYKGEEKQVDTSKIKKVWRVGKMISFTYDEGGGKTGRGAVSEKDAPKELLQMLEKQKK

SEQ ID NO: 9 - protein, 64 aa, Sulfolobus islandicus
MTTVKFKYKGEEKQVDISKIKKVWRVGKMISFTYDEGGGKTGRGAVSEKDAPKELLQMLEKQKK

SEQ ID NO: 10 - protein, 62 aa, Metallosphaera sedula.
MATKIKFKYKGQDLEVDISKVKKVWKVGKMVSFTYDDNGKTGRGAVSEKDAPKELLNMIGKK

SEQ ID NO: 11 - protein, 62 aa, Metallosphaera cuprina
MATKIKFKYKGQDLEVDISKVKKVWKVGKMVSFTYDDNGKTGRGAVSEKDAPKELLSMIGKK

SEQ ID NO: 12 - protein, 61 aa, Acidianus hospitalis
MTTVKFKYKGEEKEVDISKIKKVWRVGKMISFTYDDNGKTGRGAVSEKDAPKELLEKLEKK

SEQ ID NO: 13 - protein, 62 aa, Acidianus hospitalis
MATKVKFKYKGEEKEVDISKIKKVWRVGKMISFTYDDNGKTGRGAVSEKDAPKELLDKLEKK

SEQ ID NO: 14 - protein, 60 aa, Acidianus hospitalis
MATKVKFKYKGEEKEVDISKIKKVWRVGKMISFTYDDNGKTGRGAVSEKDAPKELLEKLK

SEQ ID NO: 15 - protein, 64 aa, Sulfurisphaera tokodaii; identical to SEQ ID NO: 6

SEQ ID NO: 16 - protein, 68 aa, Artificial Sequence
  Consensus sequence
  VARIANT (2)..(2): Xaa is V, A or T
  VARIANT (3)..(3): Xaa is T or K
  VARIANT (4)..(4): Xaa is - or K
  VARIANT (6)..(6): Xaa is R or K
  VARIANT (15)..(15): Xaa is E or Q
  VARIANT (18)..(18): Xaa is T or I
  VARIANT (31)..(31): Xaa is V or I
  VARIANT (37)..(39): Xaa Xaa Xaa is EGG or DN-
  VARIANT (57)..(57): Xaa is M or L
  VARIANT (58)..(58): Xaa is Q, D or E
  VARIANT (59)..(59): Xaa is M or K
  VARIANT (61)..(68): XaaXaaXaaXaaXaaXaaXaaXaa is -------K, EKS--GKK, EK---QKK, ARAEREKK, ARAERE-K, ARAERE--, ARA-EKKK, E-----KK or EKS--GKK
MXXXVXFKYKGEEKXVDXSKIKKVWRVGKMXSFTYDXXXGKTGRGAVSEKDAPKELXXXLXXXXXXXX

SEQ ID NO: 17 - protein, 68 aa, Artificial Sequence
  Sac7d Family consensus sequence LepR-binding protein
  VARIANT (2)..(2): Xaa is V, A or T
  VARIANT (3)..(3): Xaa is T or K
  VARIANT (4)..(4): Xaa is - or K
  VARIANT (6)..(6): Xaa is R or K
  VARIANT (8)..(8): Xaa is any amino acid
  VARIANT (9)..(9): Xaa is M, Q, T, V, I or A
  VARIANT (10)..(10): Xaa is G, A or S
  VARIANT (15)..(15): Xaa is E or Q
  VARIANT (17)..(17): Xaa is D or E
  VARIANT (18)..(18): Xaa is T or I
  VARIANT (22)..(22): Xaa is any amino acid
  VARIANT (23)..(23): Xaa is any amino acid
  VARIANT (27)..(27): Xaa is V, A, I, D or S
  VARIANT (30)..(30): Xaa is F, Y, H, M, V or A
  VARIANT (31)..(31): Xaa is V or I
  VARIANT (32)..(32): Xaa is G, A or S
  VARIANT (37)..(39): Xaa Xaa Xaa is EGG or DN-
  VARIANT (42)..(42): Xaa is T, Y, L or A
  VARIANT (44)..(44): Xaa is G, A or S
  VARIANT (48)..(48): Xaa is S, H, K, Q or R
  VARIANT (57)..(57): Xaa is M or L
  VARIANT (58)..(58): Xaa is Q, D or E
  VARIANT (59)..(59): Xaa is M or K
  VARIANT (61)..(68): XaaXaaXaaXaaXaaXaaXaaXaa is -------K, EKS--GKK, EK---QKK, ARAEREKK, ARAERE-K, ARAERE--, ARA-EKKK, E-----KK or EKS--GKK
MXXXVXFXXXGEEKXVXXSKIXXVYRXGKXXXFWYDXXXGKXGXGHVXEKDAPKELXXXLXXXXXXXX

SEQ ID NO: 18 - protein, 68 aa, Artificial Sequence
  Sac7d Family consensus sequence LepR-binding protein
  VARIANT (2)..(2): Xaa is V, A or T
  VARIANT (3)..(3): Xaa is T or K
  VARIANT (4)..(4): Xaa is - or K
  VARIANT (6)..(6): Xaa is R or K
  VARIANT (8)..(8): Xaa is any amino acid
  VARIANT (10)..(10): Xaa is G or A
  VARIANT (15)..(15): Xaa is E or Q
  VARIANT (17)..(17): Xaa is D or E
  VARIANT (18)..(18): Xaa is T or I
  VARIANT (22)..(22): Xaa is any amino acid
  VARIANT (23)..(23): Xaa is D, N, S or A
  VARIANT (27)..(27): Xaa is V, A or D
  VARIANT (30)..(30): Xaa is F, Y, H, or M
  VARIANT (31)..(31): Xaa is V or I
  VARIANT (32)..(32): Xaa is G or A
  VARIANT (37)..(39): Xaa Xaa Xaa is EGG or DN-
  VARIANT (42)..(42): Xaa is T or Y
  VARIANT (44)..(44): Xaa is G or A
  VARIANT (48)..(48): Xaa is S or K
  VARIANT (57)..(57): Xaa is M or L
  VARIANT (58)..(58): Xaa is Q, D or E
  VARIANT (59)..(59): Xaa is M or K
  VARIANT (61)..(68): XaaXaaXaaXaaXaaXaaXaaXaa is -------K, EKS--GKK, EK---QKK, ARAEREKK, ARAERE-K, ARAERE--, ARA-EKKK, E-----KK or EKS--GKK
MXXXVXFXMXGEEKXVXXSKIXXVYRXGKXXXFWYDXXXGKXGXGHVXEKDAPKELXXXLXXXXXXXX

SEQ ID NO: 19 - protein, 68 aa, Artificial Sequence
  Sac7d Family consensus sequence LepR-binding protein
  VARIANT (2)..(2): Xaa is V, A or T
  VARIANT (3)..(3): Xaa is T or K
  VARIANT (4)..(4): Xaa is - or K
  VARIANT (6)..(6): Xaa is R or K
  VARIANT (8)..(8): Xaa is any amino acid
  VARIANT (15)..(15): Xaa is E or Q
  VARIANT (17)..(17): Xaa is D or E
  VARIANT (18)..(18): Xaa is T or I
  VARIANT (22)..(22): Xaa is any amino acid
  VARIANT (23)..(23): Xaa is D, N, S or A
  VARIANT (27)..(27): Xaa is V, A or D
  VARIANT (30)..(30): Xaa is F, Y, H, or M
  VARIANT (31)..(31): Xaa is V or I
  VARIANT (37)..(39): Xaa Xaa Xaa is EGG or DN-
  VARIANT (57)..(57): Xaa is M or L
  VARIANT (58)..(58): Xaa is Q, D or E
  VARIANT (59)..(59): Xaa is M or K
  VARIANT (61)..(68): XaaXaaXaaXaaXaaXaaXaaXaa is -------K, EKS--GKK, EK---QKK, ARAEREKK, ARAERE-K, ARAERE--, ARA-EKKK, E-----KK or EKS--GKK
MXXXVXFXMGGEEKXVXXSKIXXVYRXGKXXGFWYDXXXGKTGGGHVSEKDAPKELXXXLXXXXXXXX

SEQ ID NO: 20 - protein, 68 aa, Artificial Sequence
  Sac7d Family consensus sequence LepR-binding protein F08
  VARIANT (2)..(2): Xaa is V, A or T
  VARIANT (3)..(3): Xaa is T or K
  VARIANT (4)..(4): Xaa is - or K
  VARIANT (6)..(6): Xaa is R or K
  VARIANT (15)..(15): Xaa is E or Q
  VARIANT (17)..(17): Xaa is D or E
  VARIANT (18)..(18): Xaa is T or I
  VARIANT (31)..(31): Xaa is V or I
  VARIANT (37)..(39): Xaa Xaa Xaa is EGG or DN-
  VARIANT (57)..(57): Xaa is M or L
  VARIANT (58)..(58): Xaa is Q, D or E
  VARIANT (59)..(59): Xaa is M or K
  VARIANT (61)..(68): XaaXaaXaaXaaXaaXaaXaaXaa is -------K, EKS--GKK, EK---QKK, ARAEREKK, ARAERE-K, ARAERE--, ARA-EKKK, E-----KK or EKS--GKK
MXXXVXFRMGGEEKXVXXSKIRSVYRVGKFXGFWYDXXXGKTGGGHVSEKDAPKELXXXLXXXXXXXX

SEQ ID NO: 21 - protein, 68 aa, Artificial Sequence
  Sac7d Family consensus sequence LepR-binding protein D07
  VARIANT (2)..(2): Xaa is V, A or T
  VARIANT (3)..(3): Xaa is T or K
  VARIANT (4)..(4): Xaa is - or K
  VARIANT (6)..(6): Xaa is R or K
  VARIANT (15)..(15): Xaa is E or Q
  VARIANT (17)..(17): Xaa is D or E
  VARIANT (18)..(18): Xaa is T or I
  VARIANT (31)..(31): Xaa is V or I
  VARIANT (37)..(39): Xaa Xaa Xaa is EGG or DN-
  VARIANT (57)..(57): Xaa is M or L
  VARIANT (58)..(58): Xaa is Q, D or E
  VARIANT (59)..(59): Xaa is M or K
  VARIANT (61)..(68): XaaXaaXaaXaaXaaXaaXaaXaa is -------K, EKS--GKK, EK---QKK, ARAEREKK, ARAERE-K, ARAERE--, ARA-EKKK, E-----KK or EKS--GKK
MXXXVXFVMGGEEKXVXXSKIDNVYRDGKHXGFWYDXXXGKTGGGHVSEKDAPKELXXXLXXXXXXXX

SEQ ID NO: 22 - protein, 68 aa, Artificial Sequence
  Sac7d Family consensus sequence LepR-binding protein
  VARIANT (2)..(2): Xaa is V, A or T
  VARIANT (3)..(3): Xaa is T or K
  VARIANT (4)..(4): Xaa is - or K
  VARIANT (6)..(6): Xaa is R or K
  VARIANT (8)..(8): Xaa is any amino acid
  VARIANT (9)..(9): Xaa is M, Q, T, V, I or A
  VARIANT (10)..(10): Xaa is G, A or S
  VARIANT (15)..(15): Xaa is E or Q
  VARIANT (18)..(18): Xaa is T or I
  VARIANT (22)..(22): Xaa is any amino acid
  VARIANT (23)..(23): Xaa is any amino acid
  VARIANT (27)..(27): Xaa is V, A, I, D or S
  VARIANT (30)..(30): Xaa is F, Y, H, M, V or A
  VARIANT (31)..(31): Xaa is V or I
  VARIANT (32)..(32): Xaa is G, A or S
  VARIANT (37)..(39): Xaa Xaa Xaa is EGG or DN-
  VARIANT (42)..(42): Xaa is T, Y, L or A
  VARIANT (44)..(44): Xaa is G, A or S
  VARIANT (48)..(48): Xaa is S, H, K, Q or R
  VARIANT (57)..(57): Xaa is M or L
  VARIANT (58)..(58): Xaa is Q, D or E
  VARIANT (59)..(59): Xaa is M or K
  VARIANT (61)..(68): XaaXaaXaaXaaXaaXaaXaaXaa is -------K, EKS--GKK, EK---QKK, ARAEREKK, ARAERE-K, ARAERE--, ARA-EKKK, E-----KK or EKS--GKK
MXXXVXFXXXGEEKXVDXSKIXXVYRXGKXXXFWYDXXXGKXGXGHVXEKDAPKELXXXLXXXXXXXX

SEQ ID NO: 23 - protein, 68 aa, Artificial Sequence
  Sac7d Family consensus sequence LepR-binding protein
  VARIANT (2)..(2): Xaa is V, A or T
  VARIANT (3)..(3): Xaa is T or K
  VARIANT (4)..(4): Xaa is - or K
  VARIANT (6)..(6): Xaa is R or K
  VARIANT (8)..(8): Xaa is any amino acid
  VARIANT (15)..(15): Xaa is E or Q
  VARIANT (18)..(18): Xaa is T or I
  VARIANT (22)..(22): Xaa is any amino acid
  VARIANT (23)..(23): Xaa is D, N, S or A
  VARIANT (27)..(27): Xaa is V, A or D
  VARIANT (30)..(30): Xaa is F, Y, H, or M
  VARIANT (31)..(31): Xaa is V or I
  VARIANT (37)..(39): Xaa Xaa Xaa is EGG or DN-
  VARIANT (57)..(57): Xaa is M or L
  VARIANT (58)..(58): Xaa is Q, D or E
  VARIANT (59)..(59): Xaa is M or K
  VARIANT (61)..(68): XaaXaaXaaXaaXaaXaaXaaXaa is -------K, EKS--GKK, EK---QKK, ARAEREKK, ARAERE-K, ARAERE--, ARA-EKKK, E-----KK or EKS--GKK
MXXXVXFXMGGEEKXVDXSKIXXVYRXGKXXGFWYDXXXGKTGGGHVSEKDAPKELXXXLXXXXXXXX

SEQ ID NO: 24 - protein, 68 aa, Artificial Sequence
  Sac7d Family consensus sequence LepR-binding protein F08
  VARIANT (2)..(2): Xaa is V, A or T
  VARIANT (3)..(3): Xaa is T or K
  VARIANT (4)..(4): Xaa is - or K
  VARIANT (6)..(6): Xaa is R or K
  misc_feature (15)..(15): Xaa can be any naturally occurring amino acid
  VARIANT (17)..(17): Xaa is D or E
  VARIANT (18)..(18): Xaa is T or I
  VARIANT (31)..(31): Xaa is V or I
  VARIANT (37)..(39): Xaa Xaa Xaa is EGG or DN-
  VARIANT (57)..(57): Xaa is M or L
  VARIANT (58)..(58): Xaa is Q, D or E
  VARIANT (59)..(59): Xaa is M or K
  VARIANT (61)..(68): XaaXaaXaaXaaXaaXaaXaaXaa is -------K, EKS--GKK, EK---QKK, ARAEREKK, ARAERE-K, ARAERE--, ARA-EKKK, E-----KK or EKS--GKK
MXXXVXFRMGGEEKXVDXSKIRSVYRVGKFXGFWYDXXXGKTGGGHVSEKDAPKELXXXLXXXXXXXX

SEQ ID NO: 25 - protein, 68 aa, Artificial Sequence
  Sac7d Family consensus sequence LepR-binding protein D07
  VARIANT (2)..(2): Xaa is V, A or T
  VARIANT (3)..(3): Xaa is T or K
  VARIANT (4)..(4): Xaa is - or K
  VARIANT (6)..(6): Xaa is R or K
  VARIANT (15)..(15): Xaa is E or Q
  VARIANT (18)..(18): Xaa is T or I
  VARIANT (31)..(31): Xaa is V or I
  VARIANT (37)..(39): Xaa Xaa Xaa is EGG or DN-
  VARIANT (57)..(57): Xaa is M or L
  VARIANT (58)..(58): Xaa is Q, D or E
  VARIANT (59)..(59): Xaa is M or K
  VARIANT (61)..(68): XaaXaaXaaXaaXaaXaaXaaXaa is -------K, EKS--GKK, EK---QKK, ARAEREKK, ARAERE-K, ARAERE--, ARA-EKKK, E-----KK or EKS--GKK
MXXXVXFVMGGEEKXVDXSKIDNVYRDGKHXGFWYDXXXGKTGGGHVSEKDAPKELXXXLXXXXXXXX

SEQ ID NO: 26 - protein, 68 aa, Artificial Sequence
  Sac7d Family consensus sequence LepR-binding protein
  VARIANT (2)..(2): Xaa is V, A or T
  VARIANT (3)..(3): Xaa is T or K
  VARIANT (4)..(4): Xaa is - or K
  VARIANT (6)..(6): Xaa is R or K
  VARIANT (8)..(8): Xaa is any amino acid
  VARIANT (9)..(9): Xaa is M, Q, T, V, I or A
  VARIANT (10)..(10): Xaa is G, A or S
  VARIANT (15)..(15): Xaa is E or Q
  VARIANT (18)..(18): Xaa is T or I
  VARIANT (22)..(22): Xaa is any amino acid
  VARIANT (23)..(23): Xaa is any amino acid
  VARIANT (27)..(27): Xaa is V, A, I, D or S
  VARIANT (30)..(30): Xaa is F, Y, H, M, V or A
  VARIANT (31)..(31): Xaa is V or I
  VARIANT (32)..(32): Xaa is G, A or S
  VARIANT (37)..(39): Xaa Xaa Xaa is EGG or DN-
  VARIANT (42)..(42): Xaa is T, Y, L or A
  VARIANT (44)..(44): Xaa is G, A or S
  VARIANT (48)..(48): Xaa is S, H, K, Q or R
  VARIANT (57)..(57): Xaa is M or L
  VARIANT (58)..(58): Xaa is Q, D or E
  VARIANT (59)..(59): Xaa is M or K
  VARIANT (61)..(68): XaaXaaXaaXaaXaaXaaXaaXaa is -------K, EKS--GKK, EK---QKK, ARAEREKK, ARAERE-K, ARAERE--, ARA-EKKK, E-----KK or EKS--GKK
MXXXVXFXXXGEEKXVEXSKIXXVYRXGKXXXFWYDXXXGKXGXGHVXEKDAPKELXXXLXXXXXXXX

SEQ ID NO: 27 - protein, 68 aa, Artificial Sequence
  Sac7d Family consensus sequence LepR-binding protein
  VARIANT (2)..(2): Xaa is V, A or T
  VARIANT (3)..(3): Xaa is T or K
  VARIANT (4)..(4): Xaa is - or K
  VARIANT (6)..(6): Xaa is R or K
  VARIANT (8)..(8): Xaa is any amino acid
  VARIANT (15)..(15): Xaa is E or Q
  VARIANT (18)..(18): Xaa is T or I
  VARIANT (22)..(22): Xaa is any amino acid
  VARIANT (23)..(23): Xaa is D, N, S or A
  VARIANT (27)..(27): Xaa is V, A or D
  VARIANT (30)..(30): Xaa is F, Y, H, or M
  VARIANT (31)..(31): Xaa is V or I
  VARIANT (37)..(39): Xaa Xaa Xaa is EGG or DN-
  VARIANT (57)..(57): Xaa is M or L
  VARIANT (58)..(58): Xaa is Q, D or E
  VARIANT (59)..(59): Xaa is M or K
  VARIANT (61)..(68): XaaXaaXaaXaaXaaXaaXaaXaa is -------K, EKS--GKK, EK---QKK, ARAEREKK, ARAERE-K, ARAERE--, ARA-EKKK, E-----KK or EKS--GKK
MXXXVXFXMGGEEKXVEXSKIXXVYRXGKXXGFWYDXXXGKTGGGHVSEKDAPKELXXXLXXXXXXXX

SEQ ID NO: 28 - protein, 68 aa, Artificial Sequence
  Sac7d Family consensus sequence LepR-binding protein F08
  VARIANT (2)..(2): Xaa is V, A or T
  VARIANT (3)..(3): Xaa is T or K
  VARIANT (4)..(4): Xaa is - or K
  VARIANT (6)..(6): Xaa is R or K
  misc_feature (15)..(15): Xaa can be any naturally occurring amino acid
  VARIANT (17)..(17): Xaa is D or E
  VARIANT (18)..(18): Xaa is T or I
  VARIANT (31)..(31): Xaa is V or I
  VARIANT (37)..(39): Xaa Xaa Xaa is EGG or DN-
  VARIANT (57)..(57): Xaa is M or L
  VARIANT (58)..(58): Xaa is Q, D or E
  VARIANT (59)..(59): Xaa is M or K
  VARIANT (61)..(68): XaaXaaXaaXaaXaaXaaXaaXaa is -------K, EKS--GKK, EK---QKK, ARAEREKK, ARAERE-K, ARAERE--, ARA-EKKK, E-----KK or EKS--GKK
MXXXVXFRMGGEEKXVEXSKIRSVYRVGKFXGFWYDXXXGKTGGGHVSEKDAPKELXXXLXXXXXXXX

SEQ ID NO: 29 - protein, 68 aa, Artificial Sequence
  Sac7d Family consensus sequence LepR-binding protein D07
  VARIANT (2)..(2): Xaa is V, A or T
  VARIANT (3)..(3): Xaa is T or K
  VARIANT (4)..(4): Xaa is - or K
  VARIANT (6)..(6): Xaa is R or K
  VARIANT (15)..(15): Xaa is E or Q
  VARIANT (18)..(18): Xaa is T or I
  VARIANT (31)..(31): Xaa is V or I
  VARIANT (37)..(39): Xaa Xaa Xaa is EGG or DN-
  VARIANT (57)..(57): Xaa is M or L
  VARIANT (58)..(58): Xaa is Q, D or E
  VARIANT (59)..(59): Xaa is M or K
  VARIANT (61)..(68): XaaXaaXaaXaaXaaXaaXaaXaa is -------K, EKS--GKK, EK---QKK, ARAEREKK, ARAERE-K, ARAERE--, ARA-EKKK, E-----KK or EKS--GKK
MXXXVXFVMGGEEKXVEXSKIDNVYRDGKHXGFWYDXXXGKTGGGHVSEKDAPKELXXXLXXXXXXXX

SEQ ID NO: 30 - protein, 64 aa, Artificial Sequence
  Sac7d/Aho7c consensus sequence LepR-binding protein
  VARIANT (1)..(1): Xaa is V or T
  VARIANT (6)..(6): Xaa is any amino acid
  VARIANT (7)..(7): Xaa is M, Q, T, V, I or A
  VARIANT (8)..(8): Xaa is G, A or S
  VARIANT (15)..(15): Xaa is D or E
  VARIANT (16)..(16): Xaa is T or I
  VARIANT (20)..(20): Xaa is any amino acid
  VARIANT (21)..(21): Xaa is any amino acid
  VARIANT (25)..(25): Xaa is V, A, I, D or S
  VARIANT (28)..(28): Xaa is F, Y, H, M, V or A
  VARIANT (29)..(29): Xaa is V or I
  VARIANT (30)..(30): Xaa is G, A or S
  VARIANT (36)..(36): Xaa is N or Q
  VARIANT (39)..(39): Xaa is T, Y, L or A
  VARIANT (41)..(41): Xaa is G, A or S
  VARIANT (45)..(45): Xaa is S, H, K, Q or R
  VARIANT (55)..(64): XaaXaaXaaXaaXaaXaaXaaXaaXaaXaa is DMLARAEREK, DLLARAEREK or EKLK------
XKVKFXXXGEEKEVXXSKIXXVYRXGKXXXFWYDDXGKXGXGHVXEKDAPKELLXXXXXXXXXX

SEQ ID NO: 31 - protein, 64 aa, Artificial Sequence
  Sac7d/Aho7c consensus sequence LepR-binding protein
  VARIANT (1)..(1): Xaa is V or T
  VARIANT (6)..(6): Xaa is any amino acid
  VARIANT (8)..(8): Xaa is G or A
  VARIANT (15)..(15): Xaa is D or E
  VARIANT (16)..(16): Xaa is T or I
  VARIANT (20)..(20): Xaa is any amino acid
  VARIANT (21)..(21): Xaa is D, N, S or A
  VARIANT (25)..(25): Xaa is V, A or D
  VARIANT (28)..(28): Xaa is F, Y, H, or M
  VARIANT (29)..(29): Xaa is V or I
  VARIANT (30)..(30): Xaa is G or A
  VARIANT (36)..(36): Xaa is N or Q
  VARIANT (39)..(39): Xaa is T or Y
  VARIANT (41)..(41): Xaa is G or A
  VARIANT (45)..(45): Xaa is S or K
  VARIANT (55)..(64): XaaXaaXaaXaaXaaXaaXaaXaaXaaXaa is DMLARAEREK, DLLARAEREK or EKLK------
XKVKFXMXGEEKEVXXSKIXXVYRXGKXXXFWYDDXGKXGXGHVXEKDAPKELLXXXXXXXXXX

SEQ ID NO: 32 - protein, 64 aa, Artificial Sequence
  Sac7d/Aho7c consensus sequence LepR-binding protein
  VARIANT (1)..(1): Xaa is V or T
  VARIANT (6)..(6): Xaa is any amino acid
  VARIANT (15)..(15): Xaa is D or E
  VARIANT (16)..(16): Xaa is T or I
  VARIANT (20)..(20): Xaa is any amino acid
  VARIANT (21)..(21): Xaa is D, N, S or A
  VARIANT (25)..(25): Xaa is V, A or D
  VARIANT (28)..(28): Xaa is F, Y, H, or M
  VARIANT (29)..(29): Xaa is V or I
  VARIANT (36)..(36): Xaa is N or Q
  VARIANT (55)..(64): XaaXaaXaaXaaXaaXaaXaaXaaXaaXaa is DMLARAEREK, DLLARAEREK or EKLK------
XKVKFXMGGEEKEVXXSKIXXVYRXGKXXGFWYDDXGKTGGGHVSEKDAPKELLXXXXXXXXXX

SEQ ID NO: 33 - protein, 64 aa, Artificial Sequence
  Sac7d/Aho7c consensus sequence LepR-binding protein F08
  VARIANT (1)..(1): Xaa is V or T
  VARIANT (15)..(15): Xaa is D or E
  VARIANT (16)..(16): Xaa is T or I
  VARIANT (29)..(29): Xaa is V or I
  VARIANT (36)..(36): Xaa is N or Q
  VARIANT (55)..(64): XaaXaaXaaXaaXaaXaaXaaXaaXaaXaa is DMLARAEREK, DLLARAEREK or EKLK------
XKVKFRMGGEEKEVXXSKIRSVYRVGKFXGFWYDDXGKTGGGHVSEKDAPKELLXXXXXXXXXX

SEQ ID NO: 34 - protein, 64 aa, Artificial Sequence
  Sac7d/Aho7c consensus sequence LepR-binding protein D07
  VARIANT (1)..(1): Xaa is V or T
  VARIANT (15)..(15): Xaa is D or E
  VARIANT (16)..(16): Xaa is T or I
  VARIANT (29)..(29): Xaa is V or I
  VARIANT (36)..(36): Xaa is N or Q
  VARIANT (55)..(64): XaaXaaXaaXaaXaaXaaXaaXaaXaaXaa is DMLARAEREK, DLLARAEREK or EKLK------
XKVKFVMGGEEKEVXXSKIDNVYRDGKHXGFWYDDXGKTGGGHVSEKDAPKELLXXXXXXXXXX

SEQ ID NO: 35 - protein, 64 aa, Artificial Sequence
  Sac7d based LepR-binding protein
  VARIANT (6)..(6): Xaa is any amino acid
  VARIANT (7)..(7): Xaa is M, Q, T, V, I or A
  VARIANT (8)..(8): Xaa is G, A or S
  VARIANT (15)..(15): Xaa is D or E
  VARIANT (20)..(20): Xaa is any amino acid
  VARIANT (21)..(21): Xaa is any amino acid
  VARIANT (25)..(25): Xaa is V, A, I, D or S
  VARIANT (28)..(28): Xaa is F, Y, H, M, V or A
  VARIANT (30)..(30): Xaa is G, A or S
  VARIANT (36)..(36): Xaa is N or Q
  VARIANT (39)..(39): Xaa is T, Y, L or A
  VARIANT (41)..(41): Xaa is G, A or S
  VARIANT (45)..(45): Xaa is S, H, K, Q or R
  VARIANT (56)..(56): Xaa is M or L
VKVKFXXXGEEKEVXTSKIXXVYRXGKXVXFWYDDXGKXGXGHVXEKDAPKELLDXLARAEREK

SEQ ID NO: 36 - protein, 64 aa, Artificial Sequence
  Sac7d based LepR-binding protein
  VARIANT (6)..(6): Xaa is any amino acid
  VARIANT (8)..(8): Xaa is G or A
  VARIANT (15)..(15): Xaa is D or E
  VARIANT (20)..(20): Xaa is any amino acid
  VARIANT (21)..(21): Xaa is D, N, S or A
  VARIANT (25)..(25): Xaa is V, A or D
  VARIANT (28)..(28): Xaa is F, Y, H, or M
  VARIANT (30)..(30): Xaa is G or A
  VARIANT (36)..(36): Xaa is N or Q
  VARIANT (39)..(39): Xaa is T or Y
  VARIANT (41)..(41): Xaa is G or A
  VARIANT (45)..(45): Xaa is S or K
  VARIANT (56)..(56): Xaa is M or L
VKVKFXMXGEEKEVXTSKIXXVYRXGKXVXFWYDDXGKXGXGHVXEKDAPKELLDXLARAEREK

SEQ ID NO: 37 - protein, 64 aa, Artificial Sequence
  Sac7d based LepR-binding protein
  VARIANT (6)..(6): Xaa is any amino acid
  VARIANT (15)..(15): Xaa is D or E
  VARIANT (20)..(20): Xaa is any amino acid
  VARIANT (21)..(21): Xaa is D, N, S or A
  VARIANT (25)..(25): Xaa is V, A or D
  VARIANT (28)..(28): Xaa is F, Y, H, or M
  VARIANT (36)..(36): Xaa is N or Q
  VARIANT (56)..(56): Xaa is M or L
VKVKFXMGGEEKEVXTSKIXXVYRXGKXVGFWYDDXGKTGGGHVSEKDAPKELLDXLARAEREK

SEQ ID NO: 38 - protein, 64 aa, Artificial Sequence
  Sac7d based LepR-binding protein F08
  VARIANT (15)..(15): Xaa is D or E
  VARIANT (36)..(36): Xaa is N or Q
  VARIANT (56)..(56): Xaa is M or L
VKVKFRMGGEEKEVXTSKIRSVYRVGKFVGFWYDDXGKTGGGHVSEKDAPKELLDXLARAEREK

SEQ ID NO: 39 - protein, 64 aa, Artificial Sequence
  Sac7d based LepR-binding protein D07
  VARIANT (15)..(15): Xaa is D or E
  VARIANT (36)..(36): Xaa is N or Q
  VARIANT (56)..(56): Xaa is M or L
VKVKFVMGGEEKEVXTSKIDNVYRDGKHVGFWYDDXGKTGGGHVSEKDAPKELLDXLARAEREK

SEQ ID NO: 40 - protein, 64 aa, Artificial Sequence
  Sac7d based LepR-binding protein
  VARIANT (6)..(6): Xaa is any amino acid
  VARIANT (7)..(7): Xaa is M, Q, T, V, I or A
  VARIANT (8)..(8): Xaa is G, A or S
  VARIANT (20)..(20): Xaa is any amino acid
  VARIANT (21)..(21): Xaa is any amino acid
  VARIANT (25)..(25): Xaa is V, A, I, D or S
  VARIANT (28)..(28): Xaa is F, Y, H, M, V or A
  VARIANT (30)..(30): Xaa is G, A or S
  VARIANT (39)..(39): Xaa is T, Y, L or A
  VARIANT (41)..(41): Xaa is G, A or S
  VARIANT (45)..(45): Xaa is S, H, K, Q or R
VKVKFXXXGEEKEVDTSKIXXVYRXGKXVXFWYDDNGKXGXGHVXEKDAPKELLDMLARAEREK

SEQ ID NO: 41 - protein, 64 aa, Artificial Sequence
  Sac7d based LepR-binding protein
  VARIANT (6)..(6): Xaa is any amino acid
  VARIANT (8)..(8): Xaa is G or A
  VARIANT (20)..(20): Xaa is any amino acid
  VARIANT (21)..(21): Xaa is D, N, S or A
  VARIANT (25)..(25): Xaa is V, A or D
  VARIANT (28)..(28): Xaa is F, Y, H, or M
  VARIANT (30)..(30): Xaa is G or A
  VARIANT (39)..(39): Xaa is T or Y
  VARIANT (41)..(41): Xaa is G or A
  VARIANT (45)..(45): Xaa is S or K
VKVKFXMXGEEKEVDTSKIXXVYRXGKXVXFWYDDNGKXGXGHVXEKDAPKELLDMLARAEREK

SEQ ID NO: 42 - protein, 64 aa, Artificial Sequence
  Sac7d based LepR-binding protein
  VARIANT (6)..(6): Xaa is any amino acid
  VARIANT (20)..(20): Xaa is any amino acid
  VARIANT (21)..(21): Xaa is D, N, S or A
  VARIANT (25)..(25): Xaa is V, A or D
  VARIANT (28)..(28): Xaa is F, Y, H, or M
VKVKFXMGGEEKEVDTSKIXXVYRXGKXVGFWYDDNGKTGGGHVSEKDAPKELLDMLARAEREK

SEQ ID NO: 43 - protein, 64 aa, Artificial Sequence
  Sac7d based LepR-binding protein F08
VKVKFRMGGEEKEVDTSKIRSVYRVGKFVGFWYDDNGKTGGGHVSEKDAPKELLDMLARAEREK

SEQ ID NO: 44 - protein, 64 aa, Artificial Sequence
  Sac7d based LepR-binding protein D07
VKVKFVMGGEEKEVDTSKIDNVYRDGKHVGFWYDDNGKTGGGHVSEKDAPKELLDMLARAEREK

SEQ ID NO: 45 - protein, 64 aa, Artificial Sequence
  Sac7d based LepR-binding protein
  VARIANT (6)..(6): Xaa is any amino acid
  VARIANT (7)..(7): Xaa is M, Q, T, V, I or A
  VARIANT (8)..(8): Xaa is G, A or S
  VARIANT (20)..(20): Xaa is any amino acid
  VARIANT (21)..(21): Xaa is any amino acid
  VARIANT (25)..(25): Xaa is V, A, I, D or S
  VARIANT (28)..(28): Xaa is F, Y, H, M, V or A
  VARIANT (30)..(30): Xaa is G, A or S
  VARIANT (39)..(39): Xaa is T, Y, L or A
  VARIANT (41)..(41): Xaa is G, A or S
  VARIANT (45)..(45): Xaa is S, H, K, Q or R
VKVKFXXXGEEKEVETSKIXXVYRXGKXVXFWYDDQGKXGXGHVXEKDAPKELLDLLARAEREK

SEQ ID NO: 46 - protein, 64 aa, Artificial Sequence
  Sac7d based LepR-binding protein
  VARIANT (6)..(6): Xaa is any amino acid
  VARIANT (8)..(8): Xaa is G or A
  VARIANT (20)..(20): Xaa is any amino acid
  VARIANT (21)..(21): Xaa is D, N, S or A
  VARIANT (25)..(25): Xaa is V, A or D
  VARIANT (28)..(28): Xaa is F, Y, H, or M
  VARIANT (30)..(30): Xaa is G or A
  VARIANT (39)..(39): Xaa is T or Y
  VARIANT (41)..(41): Xaa is G or A
  VARIANT (45)..(45): Xaa is S or K
VKVKFXMXGEEKEVETSKIXXVYRXGKXVXFWYDDQGKXGXGHVXEKDAPKELLDLLARAEREK

SEQ ID NO: 47 - protein, 64 aa, Artificial Sequence
  Sac7d based LepR-binding protein
  VARIANT (6)..(6): Xaa is any amino acid
  VARIANT (20)..(20): Xaa is any amino acid
  VARIANT (21)..(21): Xaa is D, N, S or A
  VARIANT (25)..(25): Xaa is V, A or D
  VARIANT (28)..(28): Xaa is F, Y, H, or M
VKVKFXMGGEEKEVETSKIXXVYRXGKXVGFWYDDQGKTGGGHVSEKDAPKELLDLLARAEREK

SEQ ID NO: 48 - protein, 64 aa, Artificial Sequence
  Sac7d based LepR-binding protein F08
VKVKFRMGGEEKEVETSKIRSVYRVGKFVGFWYDDQGKTGGGHVSEKDAPKELLDLLARAEREK

SEQ ID NO: 49 - protein, 64 aa, Artificial Sequence
  Sac7d based LepR-binding protein D07
VKVKFVMGGEEKEVETSKIDNVYRDGKHVGFWYDDQGKTGGGHVSEKDAPKELLDLLARAEREK

SEQ ID NO: 50 - protein, 58 aa, Artificial Sequence
  Aho7c based LepR-binding protein
  VARIANT (6)..(6): Xaa is any amino acid
  VARIANT (7)..(7): Xaa is M, Q, T, V, I or A
  VARIANT (8)..(8): Xaa is G, A or S
  VARIANT (15)..(15): Xaa is D or E
  VARIANT (20)..(20): Xaa is any amino acid
  VARIANT (21)..(21): Xaa is any amino acid
  VARIANT (25)..(25): Xaa is V, A, I, D or S
  VARIANT (28)..(28): Xaa is F, Y, H, M, V or A
  VARIANT (30)..(30): Xaa is G, A or S
  VARIANT (36)..(36): Xaa is N or Q
  VARIANT (39)..(39): Xaa is T, Y, L or A
  VARIANT (41)..(41): Xaa is G, A or S
  VARIANT (45)..(45): Xaa is S, H, K, Q or R
TKVKFXXXGEEKEVXISKIXXVYRXGKXIXFWYDDXGKXGXGHVXEKDAPKELLEKLK

SEQ ID NO: 51 - protein, 58 aa, Artificial Sequence
  Aho7c based LepR-binding protein
  VARIANT (6)..(6): Xaa is any amino acid
  VARIANT (8)..(8): Xaa is G or A
  VARIANT (15)..(15): Xaa is D or E
  VARIANT (20)..(20): Xaa is any amino acid
  VARIANT (21)..(21): Xaa is D, N, S or A
  VARIANT (25)..(25): Xaa is V, A or D
  VARIANT (28)..(28): Xaa is F, Y, H, or M
  VARIANT (30)..(30): Xaa is G or A
  VARIANT (36)..(36): Xaa is N or Q
  VARIANT (39)..(39): Xaa is T or Y
  VARIANT (41)..(41): Xaa is G or A
  VARIANT (45)..(45): Xaa is S or K
TKVKFXMXGEEKEVXISKIXXVYRXGKXIXFWYDDXGKXGXGHVXEKDAPKELLEKLK

SEQ ID NO: 52 - protein, 58 aa, Artificial Sequence
  Aho7c based LepR-binding protein
  VARIANT (6)..(6): Xaa is any amino acid
  VARIANT (15)..(15): Xaa is D or E
  VARIANT (20)..(20): Xaa is any amino acid
  VARIANT (21)..(21): Xaa is D, N, S or A
  VARIANT (25)..(25): Xaa is V, A or D
  VARIANT (28)..(28): Xaa is F, Y, H, or M
  VARIANT (36)..(36): Xaa is N or Q
TKVKFXMGGEEKEVXISKIXXVYRXGKXIGFWYDDXGKTGGGHVSEKDAPKELLEKLK

SEQ ID NO: 53 - protein, 58 aa, Artificial Sequence
  Aho7c based LepR-binding protein F08
  VARIANT (15)..(15): Xaa is D or E
  VARIANT (36)..(36): Xaa is N or Q
TKVKFRMGGEEKEVXISKIRSVYRVGKFIGFWYDDXGKTGGGHVSEKDAPKELLEKLK

SEQ ID NO: 54 - protein, 58 aa, Artificial Sequence
  Aho7c based LepR-binding protein D07
  VARIANT (15)..(15): Xaa is D or E
  VARIANT (36)..(36): Xaa is N or Q
TKVKFVMGGEEKEVXISKIDNVYRDGKHIGFWYDDXGKTGGGHVSEKDAPKELLEKLK

SEQ ID NO: 55 - protein, 58 aa, Artificial Sequence
  Aho7c based LepR-binding protein
  VARIANT (6)..(6): Xaa is any amino acid
  VARIANT (7)..(7): Xaa is M, Q, T, V, I or A
  VARIANT (8)..(8): Xaa is G, A or S
  VARIANT (20)..(20): Xaa is any amino acid
  VARIANT (21)..(21): Xaa is any amino acid
  VARIANT (25)..(25): Xaa is V, A, I, D or S
  VARIANT (28)..(28): Xaa is F, Y, H, M, V or A
  VARIANT (30)..(30): Xaa is G, A or S
  VARIANT (39)..(39): Xaa is T, Y, L or A
  VARIANT (41)..(41): Xaa is G, A or S
  VARIANT (45)..(45): Xaa is S, H, K, Q or R
TKVKFXXXGEEKEVDISKIXXVYRXGKXIXFWYDDNGKXGXGHVXEKDAPKELLEKLK

SEQ ID NO: 56 - protein, 58 aa, Artificial Sequence
  Aho7c based LepR-binding protein
  VARIANT (6)..(6): Xaa is any amino acid
  VARIANT (8)..(8): Xaa is G or A
  VARIANT (20)..(20): Xaa is any amino acid
  VARIANT (21)..(21): Xaa is D, N, S or A
  VARIANT (25)..(25): Xaa is V, A or D
  VARIANT (28)..(28): Xaa is F, Y, H, or M
  VARIANT (30)..(30): Xaa is G or A
  VARIANT (39)..(39): Xaa is T or Y
  VARIANT (41)..(41): Xaa is G or A
  VARIANT (45)..(45): Xaa is S or K
TKVKFXMXGEEKEVDISKIXXVYRXGKXIXFWYDDNGKXGXGHVXEKDAPKELLEKLK

SEQ ID NO: 57 - protein, 58 aa, Artificial Sequence
  Aho7c based LepR-binding protein
  VARIANT (6)..(6): Xaa is any amino acid
  VARIANT (20)..(20): Xaa is any amino acid
  VARIANT (21)..(21): Xaa is D, N, S or A
  VARIANT (25)..(25): Xaa is V, A or D
  VARIANT (28)..(28): Xaa is F, Y, H, or M
TKVKFXMGGEEKEVDISKIXXVYRXGKXIGFWYDDNGKTGGGHVSEKDAPKELLEKLK

SEQ ID NO: 58 - protein, 58 aa, Artificial Sequence
  Aho7c based LepR-binding protein F08
TKVKFRMGGEEKEVDISKIRSVYRVGKFIGFWYDDNGKTGGGHVSEKDAPKELLEKLK

SEQ ID NO: 59 - protein, 58 aa, Artificial Sequence
  Aho7c based LepR-binding protein D07
TKVKFVMGGEEKEVDISKIDNVYRDGKHIGFWYDDNGKTGGGHVSEKDAPKELLEKLK

SEQ ID NO: 60 - protein, 58 aa, Artificial Sequence
  Aho7c based LepR-binding protein
  VARIANT (6)..(6): Xaa is any amino acid
  VARIANT (7)..(7): Xaa is M, Q, T, V, I or A
  VARIANT (8)..(8): Xaa is G, A or S
  VARIANT (20)..(20): Xaa is any amino acid
  VARIANT (21)..(21): Xaa is any amino acid
  VARIANT (25)..(25): Xaa is V, A, I, D or S
  VARIANT (28)..(28): Xaa is F, Y, H, M, V or A
  VARIANT (30)..(30): Xaa is G, A or S
  VARIANT (39)..(39): Xaa is T, Y, L or A
  VARIANT (41)..(41): Xaa is G, A or S
  VARIANT (45)..(45): Xaa is S, H, K, Q or R
TKVKFXXXGEEKEVEISKIXXVYRXGKXIXFWYDDQGKXGXGHVXEKDAPKELLEKLK

SEQ ID NO: 61 - protein, 58 aa, Artificial Sequence
  Aho7c based LepR-binding protein
  VARIANT (6)..(6): Xaa is any amino acid
  VARIANT (8)..(8): Xaa is G or A
  VARIANT (20)..(20): Xaa is any amino acid
  VARIANT (21)..(21): Xaa is D, N, S or A
  VARIANT (25)..(25): Xaa is V, A or D
  VARIANT (28)..(28): Xaa is F, Y, H, or M
  VARIANT (30)..(30): Xaa is G or A
  VARIANT (39)..(39): Xaa is T or Y
  VARIANT (41)..(41): Xaa is G or A
  VARIANT (45)..(45): Xaa is S or K
TKVKFXMXGEEKEVEISKIXXVYRXGKXIXFWYDDQGKXGXGHVXEKDAPKELLEKLK

SEQ ID NO: 62 - protein, 58 aa, Artificial Sequence
  Aho7c based LepR-binding protein
  VARIANT (6)..(6): Xaa is any amino acid
  VARIANT (20)..(20): Xaa is any amino acid
  VARIANT (21)..(21): Xaa is D, N, S or A
  VARIANT (25)..(25): Xaa is V, A or D
  VARIANT (28)..(28): Xaa is F, Y, H, or M
TKVKFXMGGEEKEVEISKIXXVYRXGKXIGFWYDDQGKTGGGHVSEKDAPKELLEKLK

SEQ ID NO: 63 - protein, 58 aa, Artificial Sequence
  Aho7c based LepR-binding protein F08
TKVKFRMGGEEKEVEISKIRSVYRVGKFIGFWYDDQGKTGGGHVSEKDAPKELLEKLK

SEQ ID NO: 64 - protein, 58 aa, Artificial Sequence
  Aho7c based LepR-binding protein D07
TKVKFVMGGEEKEVEISKIDNVYRDGKHIGFWYDDQGKTGGGHVSEKDAPKELLEKLK

SEQ ID NO: 65 - protein, 64 aa, Artificial Sequence
  Consensus sequence Sac7d / Hso7c
  VARIANT (1)..(1): Xaa is V or T
  VARIANT (16)..(16): Xaa is T or I
  VARIANT (29)..(29): Xaa is V or I
  VARIANT (55)..(64): Xaa is DMLARAEREK, DLLARAEREK or EKLK------
XKVKFKYKGEEKEVDXSKIKKVWRVGKMXSFTYDDNGKTGRGAVSEKDAPKELLXXXXXXXXXX

SEQ ID NO: 66 - protein, 59 aa, Artificial
  Sso7d based LepR-binding protein
  VARIANT (4)..(4): Xaa is any amino acid
  VARIANT (5)..(5): Xaa is M, Q, T, V, I or A
  VARIANT (6)..(6): Xaa is G, A or S
  VARIANT (18)..(18): Xaa is any amino acid
  VARIANT (19)..(19): Xaa is any amino acid
  VARIANT (23)..(23): Xaa is V, A, I, D or S
  VARIANT (26)..(26): Xaa is F, Y, H, M, V or A
  VARIANT (28)..(28): Xaa is G, A or S
  VARIANT (38)..(38): Xaa is T, Y, L or A
  VARIANT (40)..(40): Xaa is G, A or S
  VARIANT (44)..(44): Xaa is S, H, K, Q or R
VKFXXXGEEKEVDISKIXXVYRXGKXIXFWYDEGGGKXGXGHVXEKDAPKELLQLLEKQ

SEQ ID NO: 67 - protein, 59 aa, Artificial
  Sso7d based LepR-binding protein
  VARIANT (4)..(4): Xaa is any amino acid
  VARIANT (6)..(6): Xaa is G or A
  VARIANT (18)..(18): Xaa is any amino acid
  VARIANT (19)..(19): Xaa is D, N, S or A
  VARIANT (23)..(23): Xaa is V, A or D
  VARIANT (26)..(26): Xaa is F, Y, H, or M
  VARIANT (28)..(28): Xaa is G or A
  VARIANT (38)..(38): Xaa is T or Y
  VARIANT (40)..(40): Xaa is G or A
  VARIANT (44)..(44): Xaa is S or K
VKFXMXGEEKEVDISKIXXVYRXGKXIXFWYDEGGGKXGXGHVXEKDAPKELLQLLEKQ

SEQ ID NO: 68 - protein, 59 aa, Artificial
  Sso7d based LepR-binding protein
  VARIANT (4)..(4): Xaa is any amino acid
  VARIANT (18)..(18): Xaa is any amino acid
  VARIANT (19)..(19): Xaa is D, N, S or A
  VARIANT (23)..(23): Xaa is V, A or D
  VARIANT (26)..(26): Xaa is F, Y, H, or M
VKFXMGGEEKEVDISKIXXVYRXGKXIGFWYDEGGGKTGGGHVSEKDAPKELLQLLEKQ

SEQ ID NO: 69 - protein, 59 aa, Artificial
  Sso7d based LepR-binding protein
VKFRMGGEEKEVDISKIRSVYRVGKFIGFWYDEGGGKTGGGHVSEKDAPKELLQLLEKQ

SEQ ID NO: 70 - protein, 59 aa, Artificial
  Sso7d based LepR-binding protein
VKFVMGGEEKEVDISKIDNVYRDGKHIGFWYDEGGGKTGGGHVSEKDAPKELLQLLEKQ

SEQ ID NO: 71 - protein, 6 aa, Artificial
  C-term of Sac7d family consensus sequence - Table 9
EKSGKK

SEQ ID NO: 72 - protein, 5 aa, Artificial
  C-term of Sac7d family consensus sequence - Table 9
EKQKK

SEQ ID NO: 73 - protein, 8 aa, Artificial
  C-term of Sac7d family consensus sequence - Table 9
ARAEREKK

SEQ ID NO: 74 - protein, 7 aa, Artificial
  C-term of Sac7d family consensus sequence - Table 9
ARAEREK

SEQ ID NO: 75 - protein, 6 aa, Artificial
  C-term of Sac7d family consensus sequence - Table 9
ARAERE

SEQ ID NO: 76 - protein, 7 aa, Artificial
  C-term of Sac7d family consensus sequence - Table 9
ARAEKKK

SEQ ID NO: 77 - protein, 6 aa, Artificial
  C-term of Sac7d family consensus sequence - Table 9
EKSGKK

SEQ ID NO: 78 - protein, 10 aa, Artificial
  C-term of Sac7d-Aho7c consensus sequence - Table 1
DMLARAEREK

SEQ ID NO: 79 - protein, 10 aa, Artificial
  C-term of Sac7d-Aho7c consensus sequence - Table 1
DLLARAEREK

SEQ ID NO: 80 - protein, 4 aa, Artificial
  C-term of Sac7d-Aho7c consensus sequence - Table 1
EKLK